European Patent Specification EP 4 172 190 B1, published January 29, 2025. Title: MODIFIED GELATINS. Applicant: FUJIFILM Corporation. The sequence listing filed with the application follows.

SEQUENCE LISTING (4 sequences)

SEQ ID NO: 1 - protein, 571 aa, Artificial Sequence
  Description of Artificial Sequence: recombinant gelatin
GAPGAPGLQGAPGLQGMPGERGAAGLPGPKGERGDAGPKGADGAPGAPGLQGMPGERGAAGLPGPKGERGDAGPKGADGAPGKDGVRGLAGPIGPPGERGAAGLPGPKGERGDAGPKGADGAPGKDGVRGLAGPIGPPGPAGAPGAPGLQGMPGERGAAGLPGPKGERGDAGPKGADGAPGKDGVRGLAGPPGAPGLQGAPGLQGMPGERGAAGLPGPKGERGDAGPKGADGAPGAPGLQGMPGERGAAGLPGPKGERGDAGPKGADGAPGKDGVRGLAGPIGPPGERGAAGLPGPKGERGDAGPKGADGAPGKDGVRGLAGPIGPPGPAGAPGAPGLQGMPGERGAAGLPGPKGERGDAGPKGADGAPGKDGVRGLAGPPGAPGLQGAPGLQGMPGERGAAGLPGPKGERGDAGPKGADGAPGAPGLQGMPGERGAAGLPGPKGERGDAGPKGADGAPGKDGVRGLAGPIGPPGERGAAGLPGPKGERGDAGPKGADGAPGKDGVRGLAGPIGPPGPAGAPGAPGLQGMPGERGAAGLPGPKGERGDAGPKGADGAPGKDGVRGLAGPPG

SEQ ID NO: 2 - protein, 949 aa, Artificial Sequence
  Description of Artificial Sequence: recombinant gelatin
GAPGAPGLQGAPGLQGMPGERGAAGLPGPKGERGDAGPKGADGAPGAPGLQGMPGERGAAGLPGPKGERGDAGPKGADGAPGKDGVRGLAGPIGPPGERGAAGLPGPKGERGDAGPKGADGAPGKDGVRGLAGPIGPPGPAGAPGAPGLQGMPGERGAAGLPGPKGERGDAGPKGADGAPGKDGVRGLAGPPGAPGLQGAPGLQGMPGERGAAGLPGPKGERGDAGPKGADGAPGAPGLQGMPGERGAAGLPGPKGERGDAGPKGADGAPGKDGVRGLAGPIGPPGERGAAGLPGPKGERGDAGPKGADGAPGKDGVRGLAGPIGPPGPAGAPGAPGLQGMPGERGAAGLPGPKGERGDAGPKGADGAPGKDGVRGLAGPPGAPGLQGAPGLQGMPGERGAAGLPGPKGERGDAGPKGADGAPGAPGLQGMPGERGAAGLPGPKGERGDAGPKGADGAPGKDGVRGLAGPIGPPGERGAAGLPGPKGERGDAGPKGADGAPGKDGVRGLAGPIGPPGPAGAPGAPGLQGMPGERGAAGLPGPKGERGDAGPKGADGAPGKDGVRGLAGPPGAPGLQGAPGLQGMPGERGAAGLPGPKGERGDAGPKGADGAPGAPGLQGMPGERGAAGLPGPKGERGDAGPKGADGAPGKDGVRGLAGPIGPPGERGAAGLPGPKGERGDAGPKGADGAPGKDGVRGLAGPIGPPGPAGAPGAPGLQGMPGERGAAGLPGPKGERGDAGPKGADGAPGKDGVRGLAGPPGAPGLQGAPGLQGMPGERGAAGLPGPKGERGDAGPKGADGAPGAPGLQGMPGERGAAGLPGPKGERGDAGPKGADGAPGKDGVRGLAGPIGPPGERGAAGLPGPKGERGDAGPKGADGAPGKDGVRGLAGPIGPPGPAGAPGAPGLQGMPGERGAAGLPGPKGERGDAGPKGADGAPGKDGVRGLAGPPG

SEQ ID NO: 3 - protein, 506 aa, Artificial Sequence
  Description of Artificial Sequence: recombinant gelatin
GPQGARGQPGVMGFPGPKGANGEPGKAGEKGLPGAPGLRGLPGKDGEAGAAGPPGPAGPAGERGEQGAPGPPGFQGLPGPPGPPGEGGKPGDQGVPGEAGAPGLVGPRGERGFPGERGAPGAQGLQGPRGLPGAPGPDGPKGAAGPAGPPGAQGPPGLQGMPGERGAAGIAGPKGDRGDVGEKGPEGAPGKDGGRGLGGPIGPPGPAGANGEKGEVGPPGPAGAAGARGAPGERGEAGPPGPAGFAGPPGADGQPGAKGEQGEAGQKGDAGAPGPQGPGGAPGPQGPAGVAGPKGARGAQGPPGAAGFPGAAGRVGPPGLQGNPGPPGPPGPAGKDGPKGARGDAGPPGRAGEPGLQGPAGPPGEKGEPGDDGPPGAEGPPGPQGLAGQRGIVGLPGQRGERGFPGLPGPAGEPGKQGAPGAAGDRGPPGPVGPPGLAGPAGEPGREGGPGADGPPGRDGAAGVKGDRGEAGAVGAPGAPGPPGAPGPAGPPGPQGDRGEAGAQGP

SEQ ID NO: 4 - protein, 821 aa, Artificial Sequence
  Description of Artificial Sequence: recombinant gelatin
GPPGEPGPTGLPGPPGERGGPGSRGFPGADGVAGPKGPAGERGSPGPAGPKGSPGEAGRPGEAGLPGAKGLTGSPGSPGPDGKTGPPGPAGQDGRPGPPGPPGARGQAGVMGFPGPKGAAGEPGKAGERGVPGPPGAVGPAGKDGEAGAQGPPGPAGPAGERGEQGPAGSPGFQGLPGPAGPPGEAGKPGEQGVPGDLGAPGPSGPAGEPGPTGLPGPPGERGGPGSRGFPGADGVAGPKGPAGERGSPGPAGPKGSPGEAGRPGEAGLPGAKGLTGSPGSPGPDGKTGPPGPAGQDGRPGPPGPPGARGQAGVMGFPGPKGAAGEPGKAGERGVPGPPGAVGPAGKDGEAGAQGPPGPAGPAGERGEQGPAGSPGFQGLPGPAGPPGEAGKPGEQGVPGDLGAPGPSGPAGEPGPTGLPGPPGERGGPGSRGFPGADGVAGPKGPAGERGSPGPAGPKGSPGEAGRPGEAGLPGAKGLTGSPGSPGPDGKTGPPGPAGQDGRPGPPGPPGARGQAGVMGFPGPKGAAGEPGKAGERGVPGPPGAVGPAGKDGEAGAQGPPGPAGPAGERGEQGPAGSPGFQGLPGPAGPPGEAGKPGEQGVPGDLGAPGPSGPAGEPGPTGLPGPPGERGGPGSRGFPGADGVAGPKGPAGERGSPGPAGPKGSPGEAGRPGEAGLPGAKGLTGSPGSPGPDGKTGPPGPAGQDGRPGPPGPPGARGQAGVMGFPGPKGAAGEPGKAGERGVPGPPGAVGPAGKDGEAGAQGPPGPAGPAGERGEQGPAGSPGFQGLPGPAGPPGEAGKPGEQGVPGDLGAPGPSGPAGG